European Patent Specification EP 3 795 681 B1, published September 18, 2024. Title: POLYMERASE COMPOSITIONS AND METHODS OF MAKING AND USING SAME. Applicant: MAZUR, Daniel TOZER, Eileen CHEN, Sihong VANDER HORN, Peter LINCECUM, Tommie. The sequence listing filed with the application follows.

SEQUENCE LISTING (44 sequences)

SEQ ID NO: 1 - protein, 832 aa, Thermus aquaticus [sequence omitted]

SEQ ID NO: 2 - protein, 832 aa, Artificial Sequence
  Synthetic:  Taq mutant E397V (Hit #1)
MRGMLPLFEPKGRVLLVDGHHLAYRTFHALKGLTTSRGEPVQAVYGFAKSLLKALKEDGDAVIVVFDAKAPSFRHEAYGGYKAGRAPTPEDFPRQLALIKELVDLLGLARLEVPGYEADDVLASLAKKAEKEGYEVRILTADKDLYQLLSDRIHVLHPEGYLITPAWLWEKYGLRPDQWADYRALTGDESDNLPGVKGIGEKTARKLLEEWGSLEALLKNLDRLKPAIREKILAHMDDLKLSWDLAKVRTDLPLEVDFAKRREPDRERLRAFLERLEFGSLLHEFGLLESPKALEEAPWPPPEGAFVGFVLSRKEPMWADLLALAAARGGRVHRAPEPYKALRDLKEARGLLAKDLSVLALREGLGLPPGDDPMLLAYLLDPSNTTPEGVARRYGGVWTEEAGERAALSERLFANLWGRLEGEERLLWLYREVERPLSAVLAHMEATGVRLDVAYLRALSLEVAEEIARLEAEVFRLAGHPFNLNSRDQLERVLFDELGLPAIGKTEKTGKRSTSAAVLEALREAHPIVEKILQYRELTKLKSTYIDPLPDLIHPRTGRLHTRFNQTATATGRLSSSDPNLQNIPVRTPLGQRIRRAFIAEEGWLLVALDYSQIELRVLAHLSGDENLIRVFQEGRDIHTETASWMFGVPREAVDPLMRRAAKTINFGVLYGMSAHRLSQELAIPYEEAQAFIERYFQSFPKVRAWIEKTLEEGRRRGYVETLFGRRRYVPDLEARVKSVREAAERMAFNMPVQGTAADLMKLAMVKLFPRLEEMGARMLLQVHDELVLEAPKERAEAVARLAKEVMEGVYPLAVPLEVEVGIGEDWLSAKE

SEQ ID NO: 3 - protein, 832 aa, Artificial Sequence
  Synthetic:  (L763F + E805I)
MRGMLPLFEPKGRVLLVDGHHLAYRTFHALKGLTTSRGEPVQAVYGFAKSLLKALKEDGDAVIVVFDAKAPSFRHEAYGGYKAGRAPTPEDFPRQLALIKELVDLLGLARLEVPGYEADDVLASLAKKAEKEGYEVRILTADKDLYQLLSDRIHVLHPEGYLITPAWLWEKYGLRPDQWADYRALTGDESDNLPGVKGIGEKTARKLLEEWGSLEALLKNLDRLKPAIREKILAHMDDLKLSWDLAKVRTDLPLEVDFAKRREPDRERLRAFLERLEFGSLLHEFGLLESPKALEEAPWPPPEGAFVGFVLSRKEPMWADLLALAAARGGRVHRAPEPYKALRDLKEARGLLAKDLSVLALREGLGLPPGDDPMLLAYLLDPSNTTPEGVARRYGGEWTEEAGERAALSERLFANLWGRLEGEERLLWLYREVERPLSAVLAHMEATGVRLDVAYLRALSLEVAEEIARLEAEVFRLAGHPFNLNSRDQLERVLFDELGLPAIGKTEKTGKRSTSAAVLEALREAHPIVEKILQYRELTKLKSTYIDPLPDLIHPRTGRLHTRFNQTATATGRLSSSDPNLQNIPVRTPLGQRIRRAFIAEEGWLLVALDYSQIELRVLAHLSGDENLIRVFQEGRDIHTETASWMFGVPREAVDPLMRRAAKTINFGVLYGMSAHRLSQELAIPYEEAQAFIERYFQSFPKVRAWIEKTLEEGRRRGYVETLFGRRRYVPDLEARVKSVREAAERMAFNMPVQGTAADLMKFAMVKLFPRLEEMGARMLLQVHDELVLEAPKERAEAVARLAKIVMEGVYPLAVPLEVEVGIGEDWLSAKE

SEQ ID NO: 4 - protein, 832 aa, Artificial Sequence
  Synthetic:  (E397V + E745T + L763F)
MRGMLPLFEPKGRVLLVDGHHLAYRTFHALKGLTTSRGEPVQAVYGFAKSLLKALKEDGDAVIVVFDAKAPSFRHEAYGGYKAGRAPTPEDFPRQLALIKELVDLLGLARLEVPGYEADDVLASLAKKAEKEGYEVRILTADKDLYQLLSDRIHVLHPEGYLITPAWLWEKYGLRPDQWADYRALTGDESDNLPGVKGIGEKTARKLLEEWGSLEALLKNLDRLKPAIREKILAHMDDLKLSWDLAKVRTDLPLEVDFAKRREPDRERLRAFLERLEFGSLLHEFGLLESPKALEEAPWPPPEGAFVGFVLSRKEPMWADLLALAAARGGRVHRAPEPYKALRDLKEARGLLAKDLSVLALREGLGLPPGDDPMLLAYLLDPSNTTPEGVARRYGGVWTEEAGERAALSERLFANLWGRLEGEERLLWLYREVERPLSAVLAHMEATGVRLDVAYLRALSLEVAEEIARLEAEVFRLAGHPFNLNSRDQLERVLFDELGLPAIGKTEKTGKRSTSAAVLEALREAHPIVEKILQYRELTKLKSTYIDPLPDLIHPRTGRLHTRFNQTATATGRLSSSDPNLQNIPVRTPLGQRIRRAFIAEEGWLLVALDYSQIELRVLAHLSGDENLIRVFQEGRDIHTETASWMFGVPREAVDPLMRRAAKTINFGVLYGMSAHRLSQELAIPYEEAQAFIERYFQSFPKVRAWIEKTLEEGRRRGYVETLFGRRRYVPDLEARVKSVREAATRMAFNMPVQGTAADLMKFAMVKLFPRLEEMGARMLLQVHDELVLEAPKERAEAVARLAKEVMEGVYPLAVPLEVEVGIGEDWLSAKE

SEQ ID NO: 5 - protein, 832 aa, Artificial Sequence
  Synthetic:  P6N
MRGMLNLFEPKGRVLLVDGHHLAYRTFHALKGLTTSRGEPVQAVYGFAKSLLKALKEDGDAVIVVFDAKAPSFRHEAYGGYKAGRAPTPEDFPRQLALIKELVDLLGLARLEVPGYEADDVLASLAKKAEKEGYEVRILTADKDLYQLLSDRIHVLHPEGYLITPAWLWEKYGLRPDQWADYRALTGDESDNLPGVKGIGEKTARKLLEEWGSLEALLKNLDRLKPAIREKILAHMDDLKLSWDLAKVRTDLPLEVDFAKRREPDRERLRAFLERLEFGSLLHEFGLLESPKALEEAPWPPPEGAFVGFVLSRKEPMWADLLALAAARGGRVHRAPEPYKALRDLKEARGLLAKDLSVLALREGLGLPPGDDPMLLAYLLDPSNTTPEGVARRYGGEWTEEAGERAALSERLFANLWGRLEGEERLLWLYREVERPLSAVLAHMEATGVRLDVAYLRALSLEVAEEIARLEAEVFRLAGHPFNLNSRDQLERVLFDELGLPAIGKTEKTGKRSTSAAVLEALREAHPIVEKILQYRELTKLKSTYIDPLPDLIHPRTGRLHTRFNQTATATGRLSSSDPNLQNIPVRTPLGQRIRRAFIAEEGWLLVALDYSQIELRVLAHLSGDENLIRVFQEGRDIHTETASWMFGVPREAVDPLMRRAAKTINFGVLYGMSAHRLSQELAIPYEEAQAFIERYFQSFPKVRAWIEKTLEEGRRRGYVETLFGRRRYVPDLEARVKSVREAAERMAFNMPVQGTAADLMKLAMVKLFPRLEEMGARMLLQVHDELVLEAPKERAEAVARLAKEVMEGVYPLAVPLEVEVGIGEDWLSAKE

SEQ ID NO: 6 - protein, 832 aa, Artificial Sequence
  Synthetic:  A77E
MRGMLPLFEPKGRVLLVDGHHLAYRTFHALKGLTTSRGEPVQAVYGFAKSLLKALKEDGDAVIVVFDAKAPSFRHEEYGGYKAGRAPTPEDFPRQLALIKELVDLLGLARLEVPGYEADDVLASLAKKAEKEGYEVRILTADKDLYQLLSDRIHVLHPEGYLITPAWLWEKYGLRPDQWADYRALTGDESDNLPGVKGIGEKTARKLLEEWGSLEALLKNLDRLKPAIREKILAHMDDLKLSWDLAKVRTDLPLEVDFAKRREPDRERLRAFLERLEFGSLLHEFGLLESPKALEEAPWPPPEGAFVGFVLSRKEPMWADLLALAAARGGRVHRAPEPYKALRDLKEARGLLAKDLSVLALREGLGLPPGDDPMLLAYLLDPSNTTPEGVARRYGGEWTEEAGERAALSERLFANLWGRLEGEERLLWLYREVERPLSAVLAHMEATGVRLDVAYLRALSLEVAEEIARLEAEVFRLAGHPFNLNSRDQLERVLFDELGLPAIGKTEKTGKRSTSAAVLEALREAHPIVEKILQYRELTKLKSTYIDPLPDLIHPRTGRLHTRFNQTATATGRLSSSDPNLQNIPVRTPLGQRIRRAFIAEEGWLLVALDYSQIELRVLAHLSGDENLIRVFQEGRDIHTETASWMFGVPREAVDPLMRRAAKTINFGVLYGMSAHRLSQELAIPYEEAQAFIERYFQSFPKVRAWIEKTLEEGRRRGYVETLFGRRRYVPDLEARVKSVREAAERMAFNMPVQGTAADLMKLAMVKLFPRLEEMGARMLLQVHDELVLEAPKERAEAVARLAKEVMEGVYPLAVPLEVEVGIGEDWLSAKE

SEQ ID NO: 7 - protein, 832 aa, Artificial Sequence
  Synthetic:  A97V
MRGMLPLFEPKGRVLLVDGHHLAYRTFHALKGLTTSRGEPVQAVYGFAKSLLKALKEDGDAVIVVFDAKAPSFRHEAYGGYKAGRAPTPEDFPRQLVLIKELVDLLGLARLEVPGYEADDVLASLAKKAEKEGYEVRILTADKDLYQLLSDRIHVLHPEGYLITPAWLWEKYGLRPDQWADYRALTGDESDNLPGVKGIGEKTARKLLEEWGSLEALLKNLDRLKPAIREKILAHMDDLKLSWDLAKVRTDLPLEVDFAKRREPDRERLRAFLERLEFGSLLHEFGLLESPKALEEAPWPPPEGAFVGFVLSRKEPMWADLLALAAARGGRVHRAPEPYKALRDLKEARGLLAKDLSVLALREGLGLPPGDDPMLLAYLLDPSNTTPEGVARRYGGEWTEEAGERAALSERLFANLWGRLEGEERLLWLYREVERPLSAVLAHMEATGVRLDVAYLRALSLEVAEEIARLEAEVFRLAGHPFNLNSRDQLERVLFDELGLPAIGKTEKTGKRSTSAAVLEALREAHPIVEKILQYRELTKLKSTYIDPLPDLIHPRTGRLHTRFNQTATATGRLSSSDPNLQNIPVRTPLGQRIRRAFIAEEGWLLVALDYSQIELRVLAHLSGDENLIRVFQEGRDIHTETASWMFGVPREAVDPLMRRAAKTINFGVLYGMSAHRLSQELAIPYEEAQAFIERYFQSFPKVRAWIEKTLEEGRRRGYVETLFGRRRYVPDLEARVKSVREAAERMAFNMPVQGTAADLMKLAMVKLFPRLEEMGARMLLQVHDELVLEAPKERAEAVARLAKEVMEGVYPLAVPLEVEVGIGEDWLSAKE

SEQ ID NO: 8 - protein, 832 aa, Artificial Sequence
  Synthetic:  L193V
MRGMLPLFEPKGRVLLVDGHHLAYRTFHALKGLTTSRGEPVQAVYGFAKSLLKALKEDGDAVIVVFDAKAPSFRHEAYGGYKAGRAPTPEDFPRQLALIKELVDLLGLARLEVPGYEADDVLASLAKKAEKEGYEVRILTADKDLYQLLSDRIHVLHPEGYLITPAWLWEKYGLRPDQWADYRALTGDESDNVPGVKGIGEKTARKLLEEWGSLEALLKNLDRLKPAIREKILAHMDDLKLSWDLAKVRTDLPLEVDFAKRREPDRERLRAFLERLEFGSLLHEFGLLESPKALEEAPWPPPEGAFVGFVLSRKEPMWADLLALAAARGGRVHRAPEPYKALRDLKEARGLLAKDLSVLALREGLGLPPGDDPMLLAYLLDPSNTTPEGVARRYGGEWTEEAGERAALSERLFANLWGRLEGEERLLWLYREVERPLSAVLAHMEATGVRLDVAYLRALSLEVAEEIARLEAEVFRLAGHPFNLNSRDQLERVLFDELGLPAIGKTEKTGKRSTSAAVLEALREAHPIVEKILQYRELTKLKSTYIDPLPDLIHPRTGRLHTRFNQTATATGRLSSSDPNLQNIPVRTPLGQRIRRAFIAEEGWLLVALDYSQIELRVLAHLSGDENLIRVFQEGRDIHTETASWMFGVPREAVDPLMRRAAKTINFGVLYGMSAHRLSQELAIPYEEAQAFIERYFQSFPKVRAWIEKTLEEGRRRGYVETLFGRRRYVPDLEARVKSVREAAERMAFNMPVQGTAADLMKLAMVKLFPRLEEMGARMLLQVHDELVLEAPKERAEAVARLAKEVMEGVYPLAVPLEVEVGIGEDWLSAKE

SEQ ID NO: 9 - protein, 832 aa, Artificial Sequence
  Synthetic:  K240I
MRGMLPLFEPKGRVLLVDGHHLAYRTFHALKGLTTSRGEPVQAVYGFAKSLLKALKEDGDAVIVVFDAKAPSFRHEAYGGYKAGRAPTPEDFPRQLALIKELVDLLGLARLEVPGYEADDVLASLAKKAEKEGYEVRILTADKDLYQLLSDRIHVLHPEGYLITPAWLWEKYGLRPDQWADYRALTGDESDNLPGVKGIGEKTARKLLEEWGSLEALLKNLDRLKPAIREKILAHMDDLILSWDLAKVRTDLPLEVDFAKRREPDRERLRAFLERLEFGSLLHEFGLLESPKALEEAPWPPPEGAFVGFVLSRKEPMWADLLALAAARGGRVHRAPEPYKALRDLKEARGLLAKDLSVLALREGLGLPPGDDPMLLAYLLDPSNTTPEGVARRYGGEWTEEAGERAALSERLFANLWGRLEGEERLLWLYREVERPLSAVLAHMEATGVRLDVAYLRALSLEVAEEIARLEAEVFRLAGHPFNLNSRDQLERVLFDELGLPAIGKTEKTGKRSTSAAVLEALREAHPIVEKILQYRELTKLKSTYIDPLPDLIHPRTGRLHTRFNQTATATGRLSSSDPNLQNIPVRTPLGQRIRRAFIAEEGWLLVALDYSQIELRVLAHLSGDENLIRVFQEGRDIHTETASWMFGVPREAVDPLMRRAAKTINFGVLYGMSAHRLSQELAIPYEEAQAFIERYFQSFPKVRAWIEKTLEEGRRRGYVETLFGRRRYVPDLEARVKSVREAAERMAFNMPVQGTAADLMKLAMVKLFPRLEEMGARMLLQVHDELVLEAPKERAEAVARLAKEVMEGVYPLAVPLEVEVGIGEDWLSAKE

SEQ ID NO: 10 - protein, 832 aa, Artificial Sequence
  Synthetic:  R266Q
MRGMLPLFEPKGRVLLVDGHHLAYRTFHALKGLTTSRGEPVQAVYGFAKSLLKALKEDGDAVIVVFDAKAPSFRHEAYGGYKAGRAPTPEDFPRQLALIKELVDLLGLARLEVPGYEADDVLASLAKKAEKEGYEVRILTADKDLYQLLSDRIHVLHPEGYLITPAWLWEKYGLRPDQWADYRALTGDESDNLPGVKGIGEKTARKLLEEWGSLEALLKNLDRLKPAIREKILAHMDDLKLSWDLAKVRTDLPLEVDFAKRREPDQERLRAFLERLEFGSLLHEFGLLESPKALEEAPWPPPEGAFVGFVLSRKEPMWADLLALAAARGGRVHRAPEPYKALRDLKEARGLLAKDLSVLALREGLGLPPGDDPMLLAYLLDPSNTTPEGVARRYGGEWTEEAGERAALSERLFANLWGRLEGEERLLWLYREVERPLSAVLAHMEATGVRLDVAYLRALSLEVAEEIARLEAEVFRLAGHPFNLNSRDQLERVLFDELGLPAIGKTEKTGKRSTSAAVLEALREAHPIVEKILQYRELTKLKSTYIDPLPDLIHPRTGRLHTRFNQTATATGRLSSSDPNLQNIPVRTPLGQRIRRAFIAEEGWLLVALDYSQIELRVLAHLSGDENLIRVFQEGRDIHTETASWMFGVPREAVDPLMRRAAKTINFGVLYGMSAHRLSQELAIPYEEAQAFIERYFQSFPKVRAWIEKTLEEGRRRGYVETLFGRRRYVPDLEARVKSVREAAERMAFNMPVQGTAADLMKLAMVKLFPRLEEMGARMLLQVHDELVLEAPKERAEAVARLAKEVMEGVYPLAVPLEVEVGIGEDWLSAKE

SEQ ID NO: 11 - protein, 832 aa, Artificial Sequence
  Synthetic:  E267T
MRGMLPLFEPKGRVLLVDGHHLAYRTFHALKGLTTSRGEPVQAVYGFAKSLLKALKEDGDAVIVVFDAKAPSFRHEAYGGYKAGRAPTPEDFPRQLALIKELVDLLGLARLEVPGYEADDVLASLAKKAEKEGYEVRILTADKDLYQLLSDRIHVLHPEGYLITPAWLWEKYGLRPDQWADYRALTGDESDNLPGVKGIGEKTARKLLEEWGSLEALLKNLDRLKPAIREKILAHMDDLKLSWDLAKVRTDLPLEVDFAKRREPDRTRLRAFLERLEFGSLLHEFGLLESPKALEEAPWPPPEGAFVGFVLSRKEPMWADLLALAAARGGRVHRAPEPYKALRDLKEARGLLAKDLSVLALREGLGLPPGDDPMLLAYLLDPSNTTPEGVARRYGGEWTEEAGERAALSERLFANLWGRLEGEERLLWLYREVERPLSAVLAHMEATGVRLDVAYLRALSLEVAEEIARLEAEVFRLAGHPFNLNSRDQLERVLFDELGLPAIGKTEKTGKRSTSAAVLEALREAHPIVEKILQYRELTKLKSTYIDPLPDLIHPRTGRLHTRFNQTATATGRLSSSDPNLQNIPVRTPLGQRIRRAFIAEEGWLLVALDYSQIELRVLAHLSGDENLIRVFQEGRDIHTETASWMFGVPREAVDPLMRRAAKTINFGVLYGMSAHRLSQELAIPYEEAQAFIERYFQSFPKVRAWIEKTLEEGRRRGYVETLFGRRRYVPDLEARVKSVREAAERMAFNMPVQGTAADLMKLAMVKLFPRLEEMGARMLLQVHDELVLEAPKERAEAVARLAKEVMEGVYPLAVPLEVEVGIGEDWLSAKE

SEQ ID NO: 12 - protein, 832 aa, Artificial Sequence
  Synthetic:  L287T
MRGMLPLFEPKGRVLLVDGHHLAYRTFHALKGLTTSRGEPVQAVYGFAKSLLKALKEDGDAVIVVFDAKAPSFRHEAYGGYKAGRAPTPEDFPRQLALIKELVDLLGLARLEVPGYEADDVLASLAKKAEKEGYEVRILTADKDLYQLLSDRIHVLHPEGYLITPAWLWEKYGLRPDQWADYRALTGDESDNLPGVKGIGEKTARKLLEEWGSLEALLKNLDRLKPAIREKILAHMDDLKLSWDLAKVRTDLPLEVDFAKRREPDRERLRAFLERLEFGSLLHEFGTLESPKALEEAPWPPPEGAFVGFVLSRKEPMWADLLALAAARGGRVHRAPEPYKALRDLKEARGLLAKDLSVLALREGLGLPPGDDPMLLAYLLDPSNTTPEGVARRYGGEWTEEAGERAALSERLFANLWGRLEGEERLLWLYREVERPLSAVLAHMEATGVRLDVAYLRALSLEVAEEIARLEAEVFRLAGHPFNLNSRDQLERVLFDELGLPAIGKTEKTGKRSTSAAVLEALREAHPIVEKILQYRELTKLKSTYIDPLPDLIHPRTGRLHTRFNQTATATGRLSSSDPNLQNIPVRTPLGQRIRRAFIAEEGWLLVALDYSQIELRVLAHLSGDENLIRVFQEGRDIHTETASWMFGVPREAVDPLMRRAAKTINFGVLYGMSAHRLSQELAIPYEEAQAFIERYFQSFPKVRAWIEKTLEEGRRRGYVETLFGRRRYVPDLEARVKSVREAAERMAFNMPVQGTAADLMKLAMVKLFPRLEEMGARMLLQVHDELVLEAPKERAEAVARLAKEVMEGVYPLAVPLEVEVGIGEDWLSAKE

SEQ ID NO: 13 - protein, 832 aa, Artificial Sequence
  Synthetic:  P291T
MRGMLPLFEPKGRVLLVDGHHLAYRTFHALKGLTTSRGEPVQAVYGFAKSLLKALKEDGDAVIVVFDAKAPSFRHEAYGGYKAGRAPTPEDFPRQLALIKELVDLLGLARLEVPGYEADDVLASLAKKAEKEGYEVRILTADKDLYQLLSDRIHVLHPEGYLITPAWLWEKYGLRPDQWADYRALTGDESDNLPGVKGIGEKTARKLLEEWGSLEALLKNLDRLKPAIREKILAHMDDLKLSWDLAKVRTDLPLEVDFAKRREPDRERLRAFLERLEFGSLLHEFGLLESTKALEEAPWPPPEGAFVGFVLSRKEPMWADLLALAAARGGRVHRAPEPYKALRDLKEARGLLAKDLSVLALREGLGLPPGDDPMLLAYLLDPSNTTPEGVARRYGGEWTEEAGERAALSERLFANLWGRLEGEERLLWLYREVERPLSAVLAHMEATGVRLDVAYLRALSLEVAEEIARLEAEVFRLAGHPFNLNSRDQLERVLFDELGLPAIGKTEKTGKRSTSAAVLEALREAHPIVEKILQYRELTKLKSTYIDPLPDLIHPRTGRLHTRFNQTATATGRLSSSDPNLQNIPVRTPLGQRIRRAFIAEEGWLLVALDYSQIELRVLAHLSGDENLIRVFQEGRDIHTETASWMFGVPREAVDPLMRRAAKTINFGVLYGMSAHRLSQELAIPYEEAQAFIERYFQSFPKVRAWIEKTLEEGRRRGYVETLFGRRRYVPDLEARVKSVREAAERMAFNMPVQGTAADLMKLAMVKLFPRLEEMGARMLLQVHDELVLEAPKERAEAVARLAKEVMEGVYPLAVPLEVEVGIGEDWLSAKE

SEQ ID NO: 14 - protein, 832 aa, Artificial Sequence
  Synthetic:  K292C
MRGMLPLFEPKGRVLLVDGHHLAYRTFHALKGLTTSRGEPVQAVYGFAKSLLKALKEDGDAVIVVFDAKAPSFRHEAYGGYKAGRAPTPEDFPRQLALIKELVDLLGLARLEVPGYEADDVLASLAKKAEKEGYEVRILTADKDLYQLLSDRIHVLHPEGYLITPAWLWEKYGLRPDQWADYRALTGDESDNLPGVKGIGEKTARKLLEEWGSLEALLKNLDRLKPAIREKILAHMDDLKLSWDLAKVRTDLPLEVDFAKRREPDRERLRAFLERLEFGSLLHEFGLLESPCALEEAPWPPPEGAFVGFVLSRKEPMWADLLALAAARGGRVHRAPEPYKALRDLKEARGLLAKDLSVLALREGLGLPPGDDPMLLAYLLDPSNTTPEGVARRYGGEWTEEAGERAALSERLFANLWGRLEGEERLLWLYREVERPLSAVLAHMEATGVRLDVAYLRALSLEVAEEIARLEAEVFRLAGHPFNLNSRDQLERVLFDELGLPAIGKTEKTGKRSTSAAVLEALREAHPIVEKILQYRELTKLKSTYIDPLPDLIHPRTGRLHTRFNQTATATGRLSSSDPNLQNIPVRTPLGQRIRRAFIAEEGWLLVALDYSQIELRVLAHLSGDENLIRVFQEGRDIHTETASWMFGVPREAVDPLMRRAAKTINFGVLYGMSAHRLSQELAIPYEEAQAFIERYFQSFPKVRAWIEKTLEEGRRRGYVETLFGRRRYVPDLEARVKSVREAAERMAFNMPVQGTAADLMKLAMVKLFPRLEEMGARMLLQVHDELVLEAPKERAEAVARLAKEVMEGVYPLAVPLEVEVGIGEDWLSAKE

SEQ ID NO: 15 - protein, 832 aa, Artificial Sequence
  Synthetic:  E295F
MRGMLPLFEPKGRVLLVDGHHLAYRTFHALKGLTTSRGEPVQAVYGFAKSLLKALKEDGDAVIVVFDAKAPSFRHEAYGGYKAGRAPTPEDFPRQLALIKELVDLLGLARLEVPGYEADDVLASLAKKAEKEGYEVRILTADKDLYQLLSDRIHVLHPEGYLITPAWLWEKYGLRPDQWADYRALTGDESDNLPGVKGIGEKTARKLLEEWGSLEALLKNLDRLKPAIREKILAHMDDLKLSWDLAKVRTDLPLEVDFAKRREPDRERLRAFLERLEFGSLLHEFGLLESPKALFEAPWPPPEGAFVGFVLSRKEPMWADLLALAAARGGRVHRAPEPYKALRDLKEARGLLAKDLSVLALREGLGLPPGDDPMLLAYLLDPSNTTPEGVARRYGGEWTEEAGERAALSERLFANLWGRLEGEERLLWLYREVERPLSAVLAHMEATGVRLDVAYLRALSLEVAEEIARLEAEVFRLAGHPFNLNSRDQLERVLFDELGLPAIGKTEKTGKRSTSAAVLEALREAHPIVEKILQYRELTKLKSTYIDPLPDLIHPRTGRLHTRFNQTATATGRLSSSDPNLQNIPVRTPLGQRIRRAFIAEEGWLLVALDYSQIELRVLAHLSGDENLIRVFQEGRDIHTETASWMFGVPREAVDPLMRRAAKTINFGVLYGMSAHRLSQELAIPYEEAQAFIERYFQSFPKVRAWIEKTLEEGRRRGYVETLFGRRRYVPDLEARVKSVREAAERMAFNMPVQGTAADLMKLAMVKLFPRLEEMGARMLLQVHDELVLEAPKERAEAVARLAKEVMEGVYPLAVPLEVEVGIGEDWLSAKE

SEQ ID NO: 16 - protein, 832 aa, Artificial Sequence
  Synthetic:  E295N
MRGMLPLFEPKGRVLLVDGHHLAYRTFHALKGLTTSRGEPVQAVYGFAKSLLKALKEDGDAVIVVFDAKAPSFRHEAYGGYKAGRAPTPEDFPRQLALIKELVDLLGLARLEVPGYEADDVLASLAKKAEKEGYEVRILTADKDLYQLLSDRIHVLHPEGYLITPAWLWEKYGLRPDQWADYRALTGDESDNLPGVKGIGEKTARKLLEEWGSLEALLKNLDRLKPAIREKILAHMDDLKLSWDLAKVRTDLPLEVDFAKRREPDRERLRAFLERLEFGSLLHEFGLLESPKALNEAPWPPPEGAFVGFVLSRKEPMWADLLALAAARGGRVHRAPEPYKALRDLKEARGLLAKDLSVLALREGLGLPPGDDPMLLAYLLDPSNTTPEGVARRYGGEWTEEAGERAALSERLFANLWGRLEGEERLLWLYREVERPLSAVLAHMEATGVRLDVAYLRALSLEVAEEIARLEAEVFRLAGHPFNLNSRDQLERVLFDELGLPAIGKTEKTGKRSTSAAVLEALREAHPIVEKILQYRELTKLKSTYIDPLPDLIHPRTGRLHTRFNQTATATGRLSSSDPNLQNIPVRTPLGQRIRRAFIAEEGWLLVALDYSQIELRVLAHLSGDENLIRVFQEGRDIHTETASWMFGVPREAVDPLMRRAAKTINFGVLYGMSAHRLSQELAIPYEEAQAFIERYFQSFPKVRAWIEKTLEEGRRRGYVETLFGRRRYVPDLEARVKSVREAAERMAFNMPVQGTAADLMKLAMVKLFPRLEEMGARMLLQVHDELVLEAPKERAEAVARLAKEVMEGVYPLAVPLEVEVGIGEDWLSAKE

SEQ ID NO: 17 - protein, 832 aa, Artificial Sequence
  Synthetic:  G418C
MRGMLPLFEPKGRVLLVDGHHLAYRTFHALKGLTTSRGEPVQAVYGFAKSLLKALKEDGDAVIVVFDAKAPSFRHEAYGGYKAGRAPTPEDFPRQLALIKELVDLLGLARLEVPGYEADDVLASLAKKAEKEGYEVRILTADKDLYQLLSDRIHVLHPEGYLITPAWLWEKYGLRPDQWADYRALTGDESDNLPGVKGIGEKTARKLLEEWGSLEALLKNLDRLKPAIREKILAHMDDLKLSWDLAKVRTDLPLEVDFAKRREPDRERLRAFLERLEFGSLLHEFGLLESPKALEEAPWPPPEGAFVGFVLSRKEPMWADLLALAAARGGRVHRAPEPYKALRDLKEARGLLAKDLSVLALREGLGLPPGDDPMLLAYLLDPSNTTPEGVARRYGGEWTEEAGERAALSERLFANLWCRLEGEERLLWLYREVERPLSAVLAHMEATGVRLDVAYLRALSLEVAEEIARLEAEVFRLAGHPFNLNSRDQLERVLFDELGLPAIGKTEKTGKRSTSAAVLEALREAHPIVEKILQYRELTKLKSTYIDPLPDLIHPRTGRLHTRFNQTATATGRLSSSDPNLQNIPVRTPLGQRIRRAFIAEEGWLLVALDYSQIELRVLAHLSGDENLIRVFQEGRDIHTETASWMFGVPREAVDPLMRRAAKTINFGVLYGMSAHRLSQELAIPYEEAQAFIERYFQSFPKVRAWIEKTLEEGRRRGYVETLFGRRRYVPDLEARVKSVREAAERMAFNMPVQGTAADLMKLAMVKLFPRLEEMGARMLLQVHDELVLEAPKERAEAVARLAKEVMEGVYPLAVPLEVEVGIGEDWLSAKE

SEQ ID NO: 18 - protein, 832 aa, Artificial Sequence
  Synthetic:  L490Q
MRGMLPLFEPKGRVLLVDGHHLAYRTFHALKGLTTSRGEPVQAVYGFAKSLLKALKEDGDAVIVVFDAKAPSFRHEAYGGYKAGRAPTPEDFPRQLALIKELVDLLGLARLEVPGYEADDVLASLAKKAEKEGYEVRILTADKDLYQLLSDRIHVLHPEGYLITPAWLWEKYGLRPDQWADYRALTGDESDNLPGVKGIGEKTARKLLEEWGSLEALLKNLDRLKPAIREKILAHMDDLKLSWDLAKVRTDLPLEVDFAKRREPDRERLRAFLERLEFGSLLHEFGLLESPKALEEAPWPPPEGAFVGFVLSRKEPMWADLLALAAARGGRVHRAPEPYKALRDLKEARGLLAKDLSVLALREGLGLPPGDDPMLLAYLLDPSNTTPEGVARRYGGEWTEEAGERAALSERLFANLWGRLEGEERLLWLYREVERPLSAVLAHMEATGVRLDVAYLRALSLEVAEEIARLEAEVFRLAGHPFNLNSRDQQERVLFDELGLPAIGKTEKTGKRSTSAAVLEALREAHPIVEKILQYRELTKLKSTYIDPLPDLIHPRTGRLHTRFNQTATATGRLSSSDPNLQNIPVRTPLGQRIRRAFIAEEGWLLVALDYSQIELRVLAHLSGDENLIRVFQEGRDIHTETASWMFGVPREAVDPLMRRAAKTINFGVLYGMSAHRLSQELAIPYEEAQAFIERYFQSFPKVRAWIEKTLEEGRRRGYVETLFGRRRYVPDLEARVKSVREAAERMAFNMPVQGTAADLMKLAMVKLFPRLEEMGARMLLQVHDELVLEAPKERAEAVARLAKEVMEGVYPLAVPLEVEVGIGEDWLSAKE

SEQ ID NO: 19 - protein, 832 aa, Artificial Sequence
  Synthetic:  A502S
MRGMLPLFEPKGRVLLVDGHHLAYRTFHALKGLTTSRGEPVQAVYGFAKSLLKALKEDGDAVIVVFDAKAPSFRHEAYGGYKAGRAPTPEDFPRQLALIKELVDLLGLARLEVPGYEADDVLASLAKKAEKEGYEVRILTADKDLYQLLSDRIHVLHPEGYLITPAWLWEKYGLRPDQWADYRALTGDESDNLPGVKGIGEKTARKLLEEWGSLEALLKNLDRLKPAIREKILAHMDDLKLSWDLAKVRTDLPLEVDFAKRREPDRERLRAFLERLEFGSLLHEFGLLESPKALEEAPWPPPEGAFVGFVLSRKEPMWADLLALAAARGGRVHRAPEPYKALRDLKEARGLLAKDLSVLALREGLGLPPGDDPMLLAYLLDPSNTTPEGVARRYGGEWTEEAGERAALSERLFANLWGRLEGEERLLWLYREVERPLSAVLAHMEATGVRLDVAYLRALSLEVAEEIARLEAEVFRLAGHPFNLNSRDQLERVLFDELGLPSIGKTEKTGKRSTSAAVLEALREAHPIVEKILQYRELTKLKSTYIDPLPDLIHPRTGRLHTRFNQTATATGRLSSSDPNLQNIPVRTPLGQRIRRAFIAEEGWLLVALDYSQIELRVLAHLSGDENLIRVFQEGRDIHTETASWMFGVPREAVDPLMRRAAKTINFGVLYGMSAHRLSQELAIPYEEAQAFIERYFQSFPKVRAWIEKTLEEGRRRGYVETLFGRRRYVPDLEARVKSVREAAERMAFNMPVQGTAADLMKLAMVKLFPRLEEMGARMLLQVHDELVLEAPKERAEAVARLAKEVMEGVYPLAVPLEVEVGIGEDWLSAKE

SEQ ID NO: 20 - protein, 832 aa, Artificial Sequence
  Synthetic:  S543V
MRGMLPLFEPKGRVLLVDGHHLAYRTFHALKGLTTSRGEPVQAVYGFAKSLLKALKEDGDAVIVVFDAKAPSFRHEAYGGYKAGRAPTPEDFPRQLALIKELVDLLGLARLEVPGYEADDVLASLAKKAEKEGYEVRILTADKDLYQLLSDRIHVLHPEGYLITPAWLWEKYGLRPDQWADYRALTGDESDNLPGVKGIGEKTARKLLEEWGSLEALLKNLDRLKPAIREKILAHMDDLKLSWDLAKVRTDLPLEVDFAKRREPDRERLRAFLERLEFGSLLHEFGLLESPKALEEAPWPPPEGAFVGFVLSRKEPMWADLLALAAARGGRVHRAPEPYKALRDLKEARGLLAKDLSVLALREGLGLPPGDDPMLLAYLLDPSNTTPEGVARRYGGEWTEEAGERAALSERLFANLWGRLEGEERLLWLYREVERPLSAVLAHMEATGVRLDVAYLRALSLEVAEEIARLEAEVFRLAGHPFNLNSRDQLERVLFDELGLPAIGKTEKTGKRSTSAAVLEALREAHPIVEKILQYRELTKLKVTYIDPLPDLIHPRTGRLHTRFNQTATATGRLSSSDPNLQNIPVRTPLGQRIRRAFIAEEGWLLVALDYSQIELRVLAHLSGDENLIRVFQEGRDIHTETASWMFGVPREAVDPLMRRAAKTINFGVLYGMSAHRLSQELAIPYEEAQAFIERYFQSFPKVRAWIEKTLEEGRRRGYVETLFGRRRYVPDLEARVKSVREAAERMAFNMPVQGTAADLMKLAMVKLFPRLEEMGARMLLQVHDELVLEAPKERAEAVARLAKEVMEGVYPLAVPLEVEVGIGEDWLSAKE

SEQ ID NO: 21 - protein, 832 aa, Artificial Sequence
  Synthetic:  D578E
MRGMLPLFEPKGRVLLVDGHHLAYRTFHALKGLTTSRGEPVQAVYGFAKSLLKALKEDGDAVIVVFDAKAPSFRHEAYGGYKAGRAPTPEDFPRQLALIKELVDLLGLARLEVPGYEADDVLASLAKKAEKEGYEVRILTADKDLYQLLSDRIHVLHPEGYLITPAWLWEKYGLRPDQWADYRALTGDESDNLPGVKGIGEKTARKLLEEWGSLEALLKNLDRLKPAIREKILAHMDDLKLSWDLAKVRTDLPLEVDFAKRREPDRERLRAFLERLEFGSLLHEFGLLESPKALEEAPWPPPEGAFVGFVLSRKEPMWADLLALAAARGGRVHRAPEPYKALRDLKEARGLLAKDLSVLALREGLGLPPGDDPMLLAYLLDPSNTTPEGVARRYGGEWTEEAGERAALSERLFANLWGRLEGEERLLWLYREVERPLSAVLAHMEATGVRLDVAYLRALSLEVAEEIARLEAEVFRLAGHPFNLNSRDQLERVLFDELGLPAIGKTEKTGKRSTSAAVLEALREAHPIVEKILQYRELTKLKSTYIDPLPDLIHPRTGRLHTRFNQTATATGRLSSSEPNLQNIPVRTPLGQRIRRAFIAEEGWLLVALDYSQIELRVLAHLSGDENLIRVFQEGRDIHTETASWMFGVPREAVDPLMRRAAKTINFGVLYGMSAHRLSQELAIPYEEAQAFIERYFQSFPKVRAWIEKTLEEGRRRGYVETLFGRRRYVPDLEARVKSVREAAERMAFNMPVQGTAADLMKLAMVKLFPRLEEMGARMLLQVHDELVLEAPKERAEAVARLAKEVMEGVYPLAVPLEVEVGIGEDWLSAKE

SEQ ID NO: 22 - protein, 832 aa, Artificial Sequence
  Synthetic:  R593G
MRGMLPLFEPKGRVLLVDGHHLAYRTFHALKGLTTSRGEPVQAVYGFAKSLLKALKEDGDAVIVVFDAKAPSFRHEAYGGYKAGRAPTPEDFPRQLALIKELVDLLGLARLEVPGYEADDVLASLAKKAEKEGYEVRILTADKDLYQLLSDRIHVLHPEGYLITPAWLWEKYGLRPDQWADYRALTGDESDNLPGVKGIGEKTARKLLEEWGSLEALLKNLDRLKPAIREKILAHMDDLKLSWDLAKVRTDLPLEVDFAKRREPDRERLRAFLERLEFGSLLHEFGLLESPKALEEAPWPPPEGAFVGFVLSRKEPMWADLLALAAARGGRVHRAPEPYKALRDLKEARGLLAKDLSVLALREGLGLPPGDDPMLLAYLLDPSNTTPEGVARRYGGEWTEEAGERAALSERLFANLWGRLEGEERLLWLYREVERPLSAVLAHMEATGVRLDVAYLRALSLEVAEEIARLEAEVFRLAGHPFNLNSRDQLERVLFDELGLPAIGKTEKTGKRSTSAAVLEALREAHPIVEKILQYRELTKLKSTYIDPLPDLIHPRTGRLHTRFNQTATATGRLSSSDPNLQNIPVRTPLGQGIRRAFIAEEGWLLVALDYSQIELRVLAHLSGDENLIRVFQEGRDIHTETASWMFGVPREAVDPLMRRAAKTINFGVLYGMSAHRLSQELAIPYEEAQAFIERYFQSFPKVRAWIEKTLEEGRRRGYVETLFGRRRYVPDLEARVKSVREAAERMAFNMPVQGTAADLMKLAMVKLFPRLEEMGARMLLQVHDELVLEAPKERAEAVARLAKEVMEGVYPLAVPLEVEVGIGEDWLSAKE

SEQ ID NO: 23 - protein, 832 aa, Artificial Sequence
  Synthetic:  L678F
MRGMLPLFEPKGRVLLVDGHHLAYRTFHALKGLTTSRGEPVQAVYGFAKSLLKALKEDGDAVIVVFDAKAPSFRHEAYGGYKAGRAPTPEDFPRQLALIKELVDLLGLARLEVPGYEADDVLASLAKKAEKEGYEVRILTADKDLYQLLSDRIHVLHPEGYLITPAWLWEKYGLRPDQWADYRALTGDESDNLPGVKGIGEKTARKLLEEWGSLEALLKNLDRLKPAIREKILAHMDDLKLSWDLAKVRTDLPLEVDFAKRREPDRERLRAFLERLEFGSLLHEFGLLESPKALEEAPWPPPEGAFVGFVLSRKEPMWADLLALAAARGGRVHRAPEPYKALRDLKEARGLLAKDLSVLALREGLGLPPGDDPMLLAYLLDPSNTTPEGVARRYGGEWTEEAGERAALSERLFANLWGRLEGEERLLWLYREVERPLSAVLAHMEATGVRLDVAYLRALSLEVAEEIARLEAEVFRLAGHPFNLNSRDQLERVLFDELGLPAIGKTEKTGKRSTSAAVLEALREAHPIVEKILQYRELTKLKSTYIDPLPDLIHPRTGRLHTRFNQTATATGRLSSSDPNLQNIPVRTPLGQRIRRAFIAEEGWLLVALDYSQIELRVLAHLSGDENLIRVFQEGRDIHTETASWMFGVPREAVDPLMRRAAKTINFGVLYGMSAHRFSQELAIPYEEAQAFIERYFQSFPKVRAWIEKTLEEGRRRGYVETLFGRRRYVPDLEARVKSVREAAERMAFNMPVQGTAADLMKLAMVKLFPRLEEMGARMLLQVHDELVLEAPKERAEAVARLAKEVMEGVYPLAVPLEVEVGIGEDWLSAKE

SEQ ID NO: 24 - protein, 832 aa, Artificial Sequence
  Synthetic:  L678T
MRGMLPLFEPKGRVLLVDGHHLAYRTFHALKGLTTSRGEPVQAVYGFAKSLLKALKEDGDAVIVVFDAKAPSFRHEAYGGYKAGRAPTPEDFPRQLALIKELVDLLGLARLEVPGYEADDVLASLAKKAEKEGYEVRILTADKDLYQLLSDRIHVLHPEGYLITPAWLWEKYGLRPDQWADYRALTGDESDNLPGVKGIGEKTARKLLEEWGSLEALLKNLDRLKPAIREKILAHMDDLKLSWDLAKVRTDLPLEVDFAKRREPDRERLRAFLERLEFGSLLHEFGLLESPKALEEAPWPPPEGAFVGFVLSRKEPMWADLLALAAARGGRVHRAPEPYKALRDLKEARGLLAKDLSVLALREGLGLPPGDDPMLLAYLLDPSNTTPEGVARRYGGEWTEEAGERAALSERLFANLWGRLEGEERLLWLYREVERPLSAVLAHMEATGVRLDVAYLRALSLEVAEEIARLEAEVFRLAGHPFNLNSRDQLERVLFDELGLPAIGKTEKTGKRSTSAAVLEALREAHPIVEKILQYRELTKLKSTYIDPLPDLIHPRTGRLHTRFNQTATATGRLSSSDPNLQNIPVRTPLGQRIRRAFIAEEGWLLVALDYSQIELRVLAHLSGDENLIRVFQEGRDIHTETASWMFGVPREAVDPLMRRAAKTINFGVLYGMSAHRTSQELAIPYEEAQAFIERYFQSFPKVRAWIEKTLEEGRRRGYVETLFGRRRYVPDLEARVKSVREAAERMAFNMPVQGTAADLMKLAMVKLFPRLEEMGARMLLQVHDELVLEAPKERAEAVARLAKEVMEGVYPLAVPLEVEVGIGEDWLSAKE

SEQ ID NO: 25 - protein, 832 aa, Artificial Sequence
  Synthetic:  S699W
MRGMLPLFEPKGRVLLVDGHHLAYRTFHALKGLTTSRGEPVQAVYGFAKSLLKALKEDGDAVIVVFDAKAPSFRHEAYGGYKAGRAPTPEDFPRQLALIKELVDLLGLARLEVPGYEADDVLASLAKKAEKEGYEVRILTADKDLYQLLSDRIHVLHPEGYLITPAWLWEKYGLRPDQWADYRALTGDESDNLPGVKGIGEKTARKLLEEWGSLEALLKNLDRLKPAIREKILAHMDDLKLSWDLAKVRTDLPLEVDFAKRREPDRERLRAFLERLEFGSLLHEFGLLESPKALEEAPWPPPEGAFVGFVLSRKEPMWADLLALAAARGGRVHRAPEPYKALRDLKEARGLLAKDLSVLALREGLGLPPGDDPMLLAYLLDPSNTTPEGVARRYGGEWTEEAGERAALSERLFANLWGRLEGEERLLWLYREVERPLSAVLAHMEATGVRLDVAYLRALSLEVAEEIARLEAEVFRLAGHPFNLNSRDQLERVLFDELGLPAIGKTEKTGKRSTSAAVLEALREAHPIVEKILQYRELTKLKSTYIDPLPDLIHPRTGRLHTRFNQTATATGRLSSSDPNLQNIPVRTPLGQRIRRAFIAEEGWLLVALDYSQIELRVLAHLSGDENLIRVFQEGRDIHTETASWMFGVPREAVDPLMRRAAKTINFGVLYGMSAHRLSQELAIPYEEAQAFIERYFQWFPKVRAWIEKTLEEGRRRGYVETLFGRRRYVPDLEARVKSVREAAERMAFNMPVQGTAADLMKLAMVKLFPRLEEMGARMLLQVHDELVLEAPKERAEAVARLAKEVMEGVYPLAVPLEVEVGIGEDWLSAKE

SEQ ID NO: 26 - protein, 832 aa, Artificial Sequence
  Synthetic:  E713W
MRGMLPLFEPKGRVLLVDGHHLAYRTFHALKGLTTSRGEPVQAVYGFAKSLLKALKEDGDAVIVVFDAKAPSFRHEAYGGYKAGRAPTPEDFPRQLALIKELVDLLGLARLEVPGYEADDVLASLAKKAEKEGYEVRILTADKDLYQLLSDRIHVLHPEGYLITPAWLWEKYGLRPDQWADYRALTGDESDNLPGVKGIGEKTARKLLEEWGSLEALLKNLDRLKPAIREKILAHMDDLKLSWDLAKVRTDLPLEVDFAKRREPDRERLRAFLERLEFGSLLHEFGLLESPKALEEAPWPPPEGAFVGFVLSRKEPMWADLLALAAARGGRVHRAPEPYKALRDLKEARGLLAKDLSVLALREGLGLPPGDDPMLLAYLLDPSNTTPEGVARRYGGEWTEEAGERAALSERLFANLWGRLEGEERLLWLYREVERPLSAVLAHMEATGVRLDVAYLRALSLEVAEEIARLEAEVFRLAGHPFNLNSRDQLERVLFDELGLPAIGKTEKTGKRSTSAAVLEALREAHPIVEKILQYRELTKLKSTYIDPLPDLIHPRTGRLHTRFNQTATATGRLSSSDPNLQNIPVRTPLGQRIRRAFIAEEGWLLVALDYSQIELRVLAHLSGDENLIRVFQEGRDIHTETASWMFGVPREAVDPLMRRAAKTINFGVLYGMSAHRLSQELAIPYEEAQAFIERYFQSFPKVRAWIEKTLEWGRRRGYVETLFGRRRYVPDLEARVKSVREAAERMAFNMPVQGTAADLMKLAMVKLFPRLEEMGARMLLQVHDELVLEAPKERAEAVARLAKEVMEGVYPLAVPLEVEVGIGEDWLSAKE

SEQ ID NO: 27 - protein, 832 aa, Artificial Sequence
  Synthetic:  V737A
MRGMLPLFEPKGRVLLVDGHHLAYRTFHALKGLTTSRGEPVQAVYGFAKSLLKALKEDGDAVIVVFDAKAPSFRHEAYGGYKAGRAPTPEDFPRQLALIKELVDLLGLARLEVPGYEADDVLASLAKKAEKEGYEVRILTADKDLYQLLSDRIHVLHPEGYLITPAWLWEKYGLRPDQWADYRALTGDESDNLPGVKGIGEKTARKLLEEWGSLEALLKNLDRLKPAIREKILAHMDDLKLSWDLAKVRTDLPLEVDFAKRREPDRERLRAFLERLEFGSLLHEFGLLESPKALEEAPWPPPEGAFVGFVLSRKEPMWADLLALAAARGGRVHRAPEPYKALRDLKEARGLLAKDLSVLALREGLGLPPGDDPMLLAYLLDPSNTTPEGVARRYGGEWTEEAGERAALSERLFANLWGRLEGEERLLWLYREVERPLSAVLAHMEATGVRLDVAYLRALSLEVAEEIARLEAEVFRLAGHPFNLNSRDQLERVLFDELGLPAIGKTEKTGKRSTSAAVLEALREAHPIVEKILQYRELTKLKSTYIDPLPDLIHPRTGRLHTRFNQTATATGRLSSSDPNLQNIPVRTPLGQRIRRAFIAEEGWLLVALDYSQIELRVLAHLSGDENLIRVFQEGRDIHTETASWMFGVPREAVDPLMRRAAKTINFGVLYGMSAHRLSQELAIPYEEAQAFIERYFQSFPKVRAWIEKTLEEGRRRGYVETLFGRRRYVPDLEARAKSVREAAERMAFNMPVQGTAADLMKLAMVKLFPRLEEMGARMLLQVHDELVLEAPKERAEAVARLAKEVMEGVYPLAVPLEVEVGIGEDWLSAKE

SEQ ID NO: 28 - protein, 832 aa, Artificial Sequence
  Synthetic:  E745T
MRGMLPLFEPKGRVLLVDGHHLAYRTFHALKGLTTSRGEPVQAVYGFAKSLLKALKEDGDAVIVVFDAKAPSFRHEAYGGYKAGRAPTPEDFPRQLALIKELVDLLGLARLEVPGYEADDVLASLAKKAEKEGYEVRILTADKDLYQLLSDRIHVLHPEGYLITPAWLWEKYGLRPDQWADYRALTGDESDNLPGVKGIGEKTARKLLEEWGSLEALLKNLDRLKPAIREKILAHMDDLKLSWDLAKVRTDLPLEVDFAKRREPDRERLRAFLERLEFGSLLHEFGLLESPKALEEAPWPPPEGAFVGFVLSRKEPMWADLLALAAARGGRVHRAPEPYKALRDLKEARGLLAKDLSVLALREGLGLPPGDDPMLLAYLLDPSNTTPEGVARRYGGEWTEEAGERAALSERLFANLWGRLEGEERLLWLYREVERPLSAVLAHMEATGVRLDVAYLRALSLEVAEEIARLEAEVFRLAGHPFNLNSRDQLERVLFDELGLPAIGKTEKTGKRSTSAAVLEALREAHPIVEKILQYRELTKLKSTYIDPLPDLIHPRTGRLHTRFNQTATATGRLSSSDPNLQNIPVRTPLGQRIRRAFIAEEGWLLVALDYSQIELRVLAHLSGDENLIRVFQEGRDIHTETASWMFGVPREAVDPLMRRAAKTINFGVLYGMSAHRLSQELAIPYEEAQAFIERYFQSFPKVRAWIEKTLEEGRRRGYVETLFGRRRYVPDLEARVKSVREAATRMAFNMPVQGTAADLMKLAMVKLFPRLEEMGARMLLQVHDELVLEAPKERAEAVARLAKEVMEGVYPLAVPLEVEVGIGEDWLSAKE

SEQ ID NO: 29 - protein, 832 aa, Artificial Sequence
  Synthetic:  L763F
MRGMLPLFEPKGRVLLVDGHHLAYRTFHALKGLTTSRGEPVQAVYGFAKSLLKALKEDGDAVIVVFDAKAPSFRHEAYGGYKAGRAPTPEDFPRQLALIKELVDLLGLARLEVPGYEADDVLASLAKKAEKEGYEVRILTADKDLYQLLSDRIHVLHPEGYLITPAWLWEKYGLRPDQWADYRALTGDESDNLPGVKGIGEKTARKLLEEWGSLEALLKNLDRLKPAIREKILAHMDDLKLSWDLAKVRTDLPLEVDFAKRREPDRERLRAFLERLEFGSLLHEFGLLESPKALEEAPWPPPEGAFVGFVLSRKEPMWADLLALAAARGGRVHRAPEPYKALRDLKEARGLLAKDLSVLALREGLGLPPGDDPMLLAYLLDPSNTTPEGVARRYGGEWTEEAGERAALSERLFANLWGRLEGEERLLWLYREVERPLSAVLAHMEATGVRLDVAYLRALSLEVAEEIARLEAEVFRLAGHPFNLNSRDQLERVLFDELGLPAIGKTEKTGKRSTSAAVLEALREAHPIVEKILQYRELTKLKSTYIDPLPDLIHPRTGRLHTRFNQTATATGRLSSSDPNLQNIPVRTPLGQRIRRAFIAEEGWLLVALDYSQIELRVLAHLSGDENLIRVFQEGRDIHTETASWMFGVPREAVDPLMRRAAKTINFGVLYGMSAHRLSQELAIPYEEAQAFIERYFQSFPKVRAWIEKTLEEGRRRGYVETLFGRRRYVPDLEARVKSVREAAERMAFNMPVQGTAADLMKFAMVKLFPRLEEMGARMLLQVHDELVLEAPKERAEAVARLAKEVMEGVYPLAVPLEVEVGIGEDWLSAKE

SEQ ID NO: 30 - protein, 832 aa, Artificial Sequence
  Synthetic:  E790G
MRGMLPLFEPKGRVLLVDGHHLAYRTFHALKGLTTSRGEPVQAVYGFAKSLLKALKEDGDAVIVVFDAKAPSFRHEAYGGYKAGRAPTPEDFPRQLALIKELVDLLGLARLEVPGYEADDVLASLAKKAEKEGYEVRILTADKDLYQLLSDRIHVLHPEGYLITPAWLWEKYGLRPDQWADYRALTGDESDNLPGVKGIGEKTARKLLEEWGSLEALLKNLDRLKPAIREKILAHMDDLKLSWDLAKVRTDLPLEVDFAKRREPDRERLRAFLERLEFGSLLHEFGLLESPKALEEAPWPPPEGAFVGFVLSRKEPMWADLLALAAARGGRVHRAPEPYKALRDLKEARGLLAKDLSVLALREGLGLPPGDDPMLLAYLLDPSNTTPEGVARRYGGEWTEEAGERAALSERLFANLWGRLEGEERLLWLYREVERPLSAVLAHMEATGVRLDVAYLRALSLEVAEEIARLEAEVFRLAGHPFNLNSRDQLERVLFDELGLPAIGKTEKTGKRSTSAAVLEALREAHPIVEKILQYRELTKLKSTYIDPLPDLIHPRTGRLHTRFNQTATATGRLSSSDPNLQNIPVRTPLGQRIRRAFIAEEGWLLVALDYSQIELRVLAHLSGDENLIRVFQEGRDIHTETASWMFGVPREAVDPLMRRAAKTINFGVLYGMSAHRLSQELAIPYEEAQAFIERYFQSFPKVRAWIEKTLEEGRRRGYVETLFGRRRYVPDLEARVKSVREAAERMAFNMPVQGTAADLMKLAMVKLFPRLEEMGARMLLQVHDELVLGAPKERAEAVARLAKEVMEGVYPLAVPLEVEVGIGEDWLSAKE

SEQ ID NO: 31 - protein, 832 aa, Artificial Sequence
  Synthetic:  E794C
MRGMLPLFEPKGRVLLVDGHHLAYRTFHALKGLTTSRGEPVQAVYGFAKSLLKALKEDGDAVIVVFDAKAPSFRHEAYGGYKAGRAPTPEDFPRQLALIKELVDLLGLARLEVPGYEADDVLASLAKKAEKEGYEVRILTADKDLYQLLSDRIHVLHPEGYLITPAWLWEKYGLRPDQWADYRALTGDESDNLPGVKGIGEKTARKLLEEWGSLEALLKNLDRLKPAIREKILAHMDDLKLSWDLAKVRTDLPLEVDFAKRREPDRERLRAFLERLEFGSLLHEFGLLESPKALEEAPWPPPEGAFVGFVLSRKEPMWADLLALAAARGGRVHRAPEPYKALRDLKEARGLLAKDLSVLALREGLGLPPGDDPMLLAYLLDPSNTTPEGVARRYGGEWTEEAGERAALSERLFANLWGRLEGEERLLWLYREVERPLSAVLAHMEATGVRLDVAYLRALSLEVAEEIARLEAEVFRLAGHPFNLNSRDQLERVLFDELGLPAIGKTEKTGKRSTSAAVLEALREAHPIVEKILQYRELTKLKSTYIDPLPDLIHPRTGRLHTRFNQTATATGRLSSSDPNLQNIPVRTPLGQRIRRAFIAEEGWLLVALDYSQIELRVLAHLSGDENLIRVFQEGRDIHTETASWMFGVPREAVDPLMRRAAKTINFGVLYGMSAHRLSQELAIPYEEAQAFIERYFQSFPKVRAWIEKTLEEGRRRGYVETLFGRRRYVPDLEARVKSVREAAERMAFNMPVQGTAADLMKLAMVKLFPRLEEMGARMLLQVHDELVLEAPKCRAEAVARLAKEVMEGVYPLAVPLEVEVGIGEDWLSAKE

SEQ ID NO: 32 - protein, 832 aa, Artificial Sequence
  Synthetic:  E805I
MRGMLPLFEPKGRVLLVDGHHLAYRTFHALKGLTTSRGEPVQAVYGFAKSLLKALKEDGDAVIVVFDAKAPSFRHEAYGGYKAGRAPTPEDFPRQLALIKELVDLLGLARLEVPGYEADDVLASLAKKAEKEGYEVRILTADKDLYQLLSDRIHVLHPEGYLITPAWLWEKYGLRPDQWADYRALTGDESDNLPGVKGIGEKTARKLLEEWGSLEALLKNLDRLKPAIREKILAHMDDLKLSWDLAKVRTDLPLEVDFAKRREPDRERLRAFLERLEFGSLLHEFGLLESPKALEEAPWPPPEGAFVGFVLSRKEPMWADLLALAAARGGRVHRAPEPYKALRDLKEARGLLAKDLSVLALREGLGLPPGDDPMLLAYLLDPSNTTPEGVARRYGGEWTEEAGERAALSERLFANLWGRLEGEERLLWLYREVERPLSAVLAHMEATGVRLDVAYLRALSLEVAEEIARLEAEVFRLAGHPFNLNSRDQLERVLFDELGLPAIGKTEKTGKRSTSAAVLEALREAHPIVEKILQYRELTKLKSTYIDPLPDLIHPRTGRLHTRFNQTATATGRLSSSDPNLQNIPVRTPLGQRIRRAFIAEEGWLLVALDYSQIELRVLAHLSGDENLIRVFQEGRDIHTETASWMFGVPREAVDPLMRRAAKTINFGVLYGMSAHRLSQELAIPYEEAQAFIERYFQSFPKVRAWIEKTLEEGRRRGYVETLFGRRRYVPDLEARVKSVREAAERMAFNMPVQGTAADLMKLAMVKLFPRLEEMGARMLLQVHDELVLEAPKERAEAVARLAKIVMEGVYPLAVPLEVEVGIGEDWLSAKE

SEQ ID NO: 33 - protein, 832 aa, Artificial Sequence
  Synthetic:  L828A
MRGMLPLFEPKGRVLLVDGHHLAYRTFHALKGLTTSRGEPVQAVYGFAKSLLKALKEDGDAVIVVFDAKAPSFRHEAYGGYKAGRAPTPEDFPRQLALIKELVDLLGLARLEVPGYEADDVLASLAKKAEKEGYEVRILTADKDLYQLLSDRIHVLHPEGYLITPAWLWEKYGLRPDQWADYRALTGDESDNLPGVKGIGEKTARKLLEEWGSLEALLKNLDRLKPAIREKILAHMDDLKLSWDLAKVRTDLPLEVDFAKRREPDRERLRAFLERLEFGSLLHEFGLLESPKALEEAPWPPPEGAFVGFVLSRKEPMWADLLALAAARGGRVHRAPEPYKALRDLKEARGLLAKDLSVLALREGLGLPPGDDPMLLAYLLDPSNTTPEGVARRYGGEWTEEAGERAALSERLFANLWGRLEGEERLLWLYREVERPLSAVLAHMEATGVRLDVAYLRALSLEVAEEIARLEAEVFRLAGHPFNLNSRDQLERVLFDELGLPAIGKTEKTGKRSTSAAVLEALREAHPIVEKILQYRELTKLKSTYIDPLPDLIHPRTGRLHTRFNQTATATGRLSSSDPNLQNIPVRTPLGQRIRRAFIAEEGWLLVALDYSQIELRVLAHLSGDENLIRVFQEGRDIHTETASWMFGVPREAVDPLMRRAAKTINFGVLYGMSAHRLSQELAIPYEEAQAFIERYFQSFPKVRAWIEKTLEEGRRRGYVETLFGRRRYVPDLEARVKSVREAAERMAFNMPVQGTAADLMKLAMVKLFPRLEEMGARMLLQVHDELVLEAPKERAEAVARLAKEVMEGVYPLAVPLEVEVGIGEDWASAKE

SEQ ID NO: 34 - protein, 832 aa, Artificial Sequence
  Synthetic:  (REF POLY) - (Taq-LR1) D732R
MRGMLPLFEPKGRVLLVDGHHLAYRTFHALKGLTTSRGEPVQAVYGFAKSLLKALKEDGDAVIVVFDAKAPSFRHEAYGGYKAGRAPTPEDFPRQLALIKELVDLLGLARLEVPGYEADDVLASLAKKAEKEGYEVRILTADKDLYQLLSDRIHVLHPEGYLITPAWLWEKYGLRPDQWADYRALTGDESDNLPGVKGIGEKTARKLLEEWGSLEALLKNLDRLKPAIREKILAHMDDLKLSWDLAKVRTDLPLEVDFAKRREPDRERLRAFLERLEFGSLLHEFGLLESPKALEEAPWPPPEGAFVGFVLSRKEPMWADLLALAAARGGRVHRAPEPYKALRDLKEARGLLAKDLSVLALREGLGLPPGDDPMLLAYLLDPSNTTPEGVARRYGGEWTEEAGERAALSERLFANLWGRLEGEERLLWLYREVERPLSAVLAHMEATGVRLDVAYLRALSLEVAEEIARLEAEVFRLAGHPFNLNSRDQLERVLFDELGLPAIGKTEKTGKRSTSAAVLEALREAHPIVEKILQYRELTKLKSTYIDPLPDLIHPRTGRLHTRFNQTATATGRLSSSDPNLQNIPVRTPLGQRIRRAFIAEEGWLLVALDYSQIELRVLAHLSGDENLIRVFQEGRDIHTETASWMFGVPREAVDPLMRRAAKTINFGVLYGMSAHRLSQELAIPYEEAQAFIERYFQSFPKVRAWIEKTLEEGRRRGYVETLFGRRRYVPRLEARVKSVREAAERMAFNMPVQGTAADLMKLAMVKLFPRLEEMGARMLLQVHDELVLEAPKERAEAVARLAKEVMEGVYPLAVPLEVEVGIGEDWLSAKE

SEQ ID NO: 35 - protein, 6 aa, Artificial Sequence
  Synthetic peptide
  misc_feature (2)..(2): Xaa can be any naturally occurring amino acid
  misc_feature (4)..(5): Xaa can be any naturally occurring amino acid
DXSXXE

SEQ ID NO: 36 - protein, 9 aa, Artificial Sequence
  Synthetic peptide
  misc_feature (2)..(7): Xaa can be any naturally occurring amino acid
KXXXXXXYG

SEQ ID NO: 37 - protein, 4 aa, Artificial Sequence
  Synthetic peptide
VHDE

SEQ ID NO: 38 - protein, 8 aa, Artificial Sequence
  Synthetic peptide
  misc_feature (2)..(3): Xaa can be any naturally occurring amino acid
DXXSLYPS

SEQ ID NO: 39 - protein, 9 aa, Artificial Sequence
  Synthetic peptide
  misc_feature (2)..(4): Xaa can be any naturally occurring amino acid
  misc_feature (7)..(7): Xaa can be any naturally occurring amino acid
KXXXNSXYG

SEQ ID NO: 40 - protein, 6 aa, Artificial Sequence
  Synthetic peptide
YGDTDS

SEQ ID NO: 41 - protein, 6 aa, Artificial Sequence
  Synthetic peptide
  misc_feature (2)..(5): Xaa can be any naturally occurring amino acid
  misc_feature (6)..(6): Xaa is Phe or Tyr
DXXXXX

SEQ ID NO: 42 - protein, 7 aa, Artificial Sequence
  Synthetic peptide
  misc_feature (2)..(2): Xaa can be any naturally occurring amino acid
  misc_feature (4)..(6): Xaa can be any naturally occurring amino acid
  misc_feature (7)..(7): Xaa is Ser or Ala
FXGXXXX

SEQ ID NO: 43 - protein, 4 aa, Artificial Sequence
  Synthetic peptide
  misc_feature (2)..(2): Xaa can be any naturally occurring amino acid
YXDD

SEQ ID NO: 44 - protein, 9 aa, Artificial Sequence
  Synthetic peptide
  misc_feature (2)..(8): Xaa can be any naturally occurring amino acid
GXXXXXXXK